European Patent Specification EP 3 592 137 B1, published August 7, 2024. Title: RIBOSWITCH MODULATED GENE THERAPY FOR RETINAL DISEASES. Applicant: Medical College of Wisconsin Lipinski, Daniel  M Reid, Chris A. The sequence listing filed with the application follows.

SEQUENCE LISTING (79 sequences)

SEQ ID NO: 1 - DNA, 215 bp, Artificial Sequence
  synthetic
cgtatcagcaggtcccataagctttcgacaattaacgagtgtgtactcgttctatcatctcacagttaaagtcgggagaataggagccgcacgggtcctgataccagcgtgagcggagagaatcttctttctgtctattagtgaagccacagatgtaatagacagaaagaagattctctccgcctacgcccttggcagcaccgtacggttcgatc

SEQ ID NO: 2 - DNA, 121 bp, Artificial Sequence
  synthetic
ctagcgagagaatcttctttctgtctataaaagagagaatcttctttctgtctataaaagagagaatcttctttctgtctataaaagagagaatcttctttctgtctatgtcgaccctgca

SEQ ID NO: 3 - DNA, 286 bp, Artificial Sequence
  synthetic
ggttggccactccctctctgcgcgctcgctcgctcactgaggccgggcgaccaaaggtcgcccgacgcccgggctttgcccgggcggcctcagtgagcgagcgagcgcgcagagagggagtggccaactccatcactaggggtacccctagtgatggagttggccactccctctctgcgcgctcgctcgctcactgaggccgcccgggcaaagcccgggcgtcgggcgacctttggtcgcccggcctcagtgagcgagcgagcgcgcagagagggagtggccaacc

SEQ ID NO: 4 - DNA, 236 bp, Artificial Sequence
  synthetic
tcgactagagctcgctgatcagcctcgactgtgccttctagttgccagccatctgttgtttgcccctcccccgtgccttccttgaccctggaaggtgccactcccactgtcctttcctaataaaatgaggaaattgcatcgcattgtctgagtaggtgtcattctattctggggggtggggtggggcaggacagcaagggggaggattgggaagacaatagcaggcatgctgggga

SEQ ID NO: 5 - DNA, 202 bp, Artificial Sequence
  synthetic
ggtgagcgggcgggacggcccttctcctccgggctgtaattagcgcttggtttaatgacggcttgtttcttttctgtggctgcgtgaaagccttgaggggctccgggagctagagcctctgctaaccatgttcatgccttcttctttttcctacagctcctgggcaacgtgctggttattgtgctgtctcatcattttggca

SEQ ID NO: 6 - DNA, 255 bp, Artificial Sequence
  synthetic
catggtcgaggtgagccccacgttctgcttcactctccccatctcccccccctccccacccccaattttgtatttatttattttttaattattttgtgcagcgatgggggcggggggggggggggggcgcgcgccaggcggggcggggcggggcgaggggcggggcggggcgaggcggagaggtgcggcggcagccaatcagagcggcgcgctccgaaagtttccttttatggcgaggcggcggcggcggcggcc

SEQ ID NO: 7 - DNA, 255 bp, Artificial Sequence
  synthetic
aattcggtacccctagttattaatagtaatcaattacggggtcattagttcatagcccatatatggagttccgcgttacataacttacggtaaatggcccgcctggctgaccgcccaacgacccccgcccattgacgtcaataatgacgtatgttcccatagtaacgccaatagggactttccattgacgtcaatgggtggactatttacggtaaactgcccacttggcagtacatcaagtgtatcatatgccaa

SEQ ID NO: 8 - DNA, 1374 bp, Artificial Sequence
  synthetic
atggtatcatattgggacacaggagtcctcctgtgcgcccttttgagctgtcttttgctgacgggttcttcttcaggttctgataccgggagaccattcgttgaaatgtatagtgagatacccgaaattatacatatgactgaagggcgcgagctcgtcataccctgtcgggtaacaagtccaaacataacagtgaccctgaagaagttccctttggatactctcattcccgacgggaagcgaataatttgggactcaaggaagggatttatcatatctaatgcaacatataaggaaatagggctcctcacatgcgaagccacagtcaacgggcacctctacaaaactaattacctgacccatcgacagacaaataccatcattgatgtggttctgagtccatctcatggaatagagttgagtgtaggggagaagcttgttctcaattgcacagctagaaccgagttgaacgtgggtatcgattttaactgggaatacccatctagtaagcaccaacacaaaaaacttgtcaatcgagatttgaaaactcaatctggtagcgagatgaaaaagttcctgtcaactcttacaatcgatggcgtgacccggagtgatcaaggattgtatacctgcgccgccagctctggcctgatgactaaaaagaacagcacctttgtacgagtgcatgaaaaggataagactcatacatgccctccttgtcccgctccagagctgctgggaggtcccagtgttttcctcttcccaccaaagcccaaagatactctgatgattagccggacccctgaggtgacttgcgtcgtggtggatgtttcacatgaagatccagaagtgaagttcaattggtacgttgatggtgtggaggtacacaatgccaagactaaacctcgggaggaacagtataacagcacttacagagttgtcagcgtactcacagtgcttcatcaggactggttgaatggtaaggagtataagtgcaaagtgagtaataaggctctgccagcacccatagagaagacaatctcaaaggccaaaggccagccccgagaaccacaagtatacacactgccacctagtagagacgagttgacaaaaaatcaggtcagcctcacctgtctcgtgaaaggcttctaccctagcgacattgccgtagaatgggaaagcaacgggcaaccagaaaacaattataagacaacacctcccgttctcgatagtgacggaagtttcttcctgtatagcaaacttaccgtggataaatcaagatggcagcaaggtaatgtgtttagctgttcagtaatgcacgaagctctgcataaccactacacccaaaaatctttgtctctgtctccagggtga

SEQ ID NO: 9 - DNA, 3325 bp, Artificial Sequence
  synthetic
ggttggccactccctctctgcgcgctcgctcgctcactgaggccgggcgaccaaaggtcgcccgacgcccgggctttgcccgggcggcctcagtgagcgagcgagcgcgcagagagggagtggccaactccatcactaggggttcctagatctgaattcggtacccctagttattaatagtaatcaattacggggtcattagttcatagcccatatatggagttccgcgttacataacttacggtaaatggcccgcctggctgaccgcccaacgacccccgcccattgacgtcaataatgacgtatgttcccatagtaacgccaatagggactttccattgacgtcaatgggtggactatttacggtaaactgcccacttggcagtacatcaagtgtatcatatgccaagtacgccccctattgacgtcaatgacggtaaatggcccgcctggcattatgcccagtacatgaccttatgggactttcctacttggcagtacatctacgtattagtcatcgctattaccatggtcgaggtgagccccacgttctgcttcactctccccatctcccccccctccccacccccaattttgtatttatttattttttaattattttgtgcagcgatgggggcggggggggggggggggcgcgcgccaggcggggcggggcggggcgaggggcggggcggggcgaggcggagaggtgcggcggcagccaatcagagcggcgcgctccgaaagtttccttttatggcgaggcggcggcggcggcggccctataaaaagcgaagcgcgcggcgggcgggagtcgctgcgacgctgccttcgccccgtgccccgctccgccgccgcctcgcgccgcccgccccggctctgactgaccgcgttactcccacaggtgagcgggcgggacggcccttctcctccgggctgtaattagcgcttggtttaatgacggcttgtttcttttctgtggctgcgtgaaagccttgaggggctccgggagctagagcctctgctaaccatgttcatgccttcttctttttcctacagctcctgggcaacgtgctggttattgtgctgtctcatcattttggcaaagaattcctcgaagatctaggcaacgcgtattgggatctcgaggcggccgcgccgccaccctagcgagagaatcttctttctgtctataaaagagagaatcttctttctgtctataaaagagagaatcttctttctgtctataaaagagagaatcttctttctgtctatgtcgaccctgcaatggtatcatattgggacacaggagtcctcctgtgcgcccttttgagctgtcttttgctgacgggttcttcttcaggttctgataccgggagaccattcgttgaaatgtatagtgagatacccgaaattatacatatgactgaagggcgcgagctcgtcataccctgtcgggtaacaagtccaaacataacagtgaccctgaagaagttccctttggatactctcattcccgacgggaagcgaataatttgggactcaaggaagggatttatcatatctaatgcaacatataaggaaatagggctcctcacatgcgaagccacagtcaacgggcacctctacaaaactaattacctgacccatcgacagacaaataccatcattgatgtggttctgagtccatctcatggaatagagttgagtgtaggggagaagcttgttctcaattgcacagctagaaccgagttgaacgtgggtatcgattttaactgggaatacccatctagtaagcaccaacacaaaaaacttgtcaatcgagatttgaaaactcaatctggtagcgagatgaaaaagttcctgtcaactcttacaatcgatggcgtgacccggagtgatcaaggattgtatacctgcgccgccagctctggcctgatgactaaaaagaacagcacctttgtacgagtgcatgaaaaggataagactcatacatgccctccttgtcccgctccagagctgctgggaggtcccagtgttttcctcttcccaccaaagcccaaagatactctgatgattagccggacccctgaggtgacttgcgtcgtggtggatgtttcacatgaagatccagaagtgaagttcaattggtacgttgatggtgtggaggtacacaatgccaagactaaacctcgggaggaacagtataacagcacttacagagttgtcagcgtactcacagtgcttcatcaggactggttgaatggtaaggagtataagtgcaaagtgagtaataaggctctgccagcacccatagagaagacaatctcaaaggccaaaggccagccccgagaaccacaagtatacacactgccacctagtagagacgagttgacaaaaaatcaggtcagcctcacctgtctcgtgaaaggcttctaccctagcgacattgccgtagaatgggaaagcaacgggcaaccagaaaacaattataagacaacacctcccgttctcgatagtgacggaagtttcttcctgtatagcaaacttaccgtggataaatcaagatggcagcaaggtaatgtgtttagctgttcagtaatgcacgaagctctgcataaccactacacccaaaaatctttgtctctgtctccagggtgagcgtatcagcaggtcccataagctttcgacaattaacgagtgtgtactcgttctatcatctcacagttaaagtcgggagaataggagccgcacgggtcctgataccagcgtgagcggagagaatcttctttctgtctattagtgaagccacagatgtaatagacagaaagaagattctctccgcctacgcccttggcagcaccgtacggttcgatcagcttattggtacatgataagtctcaggcatcgtacgatgtcgacctgcaggagtcggtcgactagagctcgctgatcagcctcgactgtgccttctagttgccagccatctgttgtttgcccctcccccgtgccttccttgaccctggaaggtgccactcccactgtcctttcctaataaaatgaggaaattgcatcgcattgtctgagtaggtgtcattctattctggggggtggggtggggcaggacagcaagggggaggattgggaagacaatagcaggcatgctggggagagatctaggaacccctagtgatggagttggccactccctctctgcgcgctcgctcgctcactgaggccgcccgggcaaagcccgggcgtcgggcgacctttggtcgcccggcctcagtgagcgagcgagcgcgcagagagggagtggccaacc

SEQ ID NO: 10 - DNA, 27 bp, Artificial Sequence
  synthetic
gagagaatcttctttctgtctataaaa

SEQ ID NO: 11 - DNA, 168 bp, Artificial Sequence
  synthetic
ctcgaggcgatcgcaaacaaacaaagctgtcaccggatgtgctttccggtctgatgagtccgttgtccaataccagcatcgtcttgatgcccttggcagtggatggggacggaggacgaaacagcaaaaagaaaaataaaaattttttttttaattaatcttgggccc

SEQ ID NO: 12 - DNA, 175 bp, Artificial Sequence
  synthetic
ctcgaggcgatcgcaaacaaacaaagctgtcaccggatgtgctttccggtctgatgagtccgttgtccaaaacataccagatttcgatctggagaggtgaagaattcgaccacctggacgaggacggaggacgaaacagcaaaaagaaaaataaaaattaattaatcttgggccc

SEQ ID NO: 13 - DNA, 139 bp, Artificial Sequence
  synthetic
atggccggcatggtcccagcctcctcgctggcgccggctgggcaaccacataccagccgaaaggcccttggcaggtgggcgaatgggacgcacaaatctctctagcttcccagagagaagcgagagaaaagtggctctc

SEQ ID NO: 14 - DNA, 135 bp, Artificial Sequence
  synthetic
atggccggcatggtcccagcctcctcgctggcgccggctgggcaatgctataatcgcgtggatatggcacgcaagtttctaccgggcaccgtaaatgtccgactagtagcgaatgggacgcacaaatctctctag

SEQ ID NO: 15 - DNA, 134 bp, Artificial Sequence
  synthetic
caaacaaacaaaggcgcgtcctggattcgtggtaaaacataccagatttcgatctggagaggtgaagaatacgaccacctgtagtatccagctgatgagtcccaaataggacgaaacgcgctaaacaaacaaac

SEQ ID NO: 16 - DNA, 123 bp, Artificial Sequence
  synthetic
ctgaggtgcaggtacatccagctgacgagtcccaaataggacgaaagggagaggtgaagaatacgaccacctaggctcgaaagagcctaaaacatacctttcctggattccactgctatccac

SEQ ID NO: 17 - DNA, 286 bp, Artificial Sequence
  synthetic
ctagcacgggtccctaaaacataccgtgagcgcgaaagcgcccccattttgagttagtgaagccacagatgtaactcaaaatgggggcgctttcccgcctacggagaggtgaagaatacgaccacctagaagcttattggtacatgataacaccccaaaatcgaagcacttcaaaaacaccccaaaatcgaagcacttcaaaaacaccccaaaatcgaagcacttcaaaaacaccccaaaatcgaagcacttcagtctcaggcatcgtacgatgtcgacctgcagg

SEQ ID NO: 18 - DNA, 1376 bp, Artificial Sequence
  synthetic
  modified_base (1)..(1): SLIM regulatory element
  modified_base (1376)..(1376): SLIM regulatory element
aatgtccatgttgttctacactctgatcacagcttttctgatcggcatacaggcggaaccacactcagtctgataccgggagaccattcgttgaaatgtatagtgagatacccgaaattatacatatgactgaagggcgcgagctcgtcataccctgtcgggtaacaagtccaaacataacagtgaccctgaagaagttccctttggatactctcattcccgacgggaagcgaataatttgggactcaaggaagggatttatcatatctaatgcaacatataaggaaatagggctcctcacatgcgaagccacagtcaacgggcacctctacaaaactaattacctgacccatcgacagacaaataccatcattgatgtggttctgagtccatctcatggaatagagttgagtgtaggggagaagcttgttctcaattgcacagctagaaccgagttgaacgtgggtatcgattttaactgggaatacccatctagtaagcaccaacacaaaaaacttgtcaatcgagatttgaaaactcaatctggtagcgagatgaaaaagttcctgtcaactcttacaatcgatggcgtgacccggagtgatcaaggattgtatacctgcgccgccagctctggcctgatgactaaaaagaacagcacctttgtacgagtgcatgaaaaggataagactcatacatgccctccttgtcccgctccagagctgctgggaggtcccagtgttttcctcttcccaccaaagcccaaagatactctgatgattagccggacccctgaggtgacttgcgtcgtggtggatgtttcacatgaagatccagaagtgaagttcaattggtacgttgatggtgtggaggtacacaatgccaagactaaacctcgggaggaacagtataacagcacttacagagttgtcagcgtactcacagtgcttcatcaggactggttgaatggtaaggagtataagtgcaaagtgagtaataaggctctgccagcacccatagagaagacaatctcaaaggccaaaggccagccccgagaaccacaagtatacacactgccacctagtagagacgagttgacaaaaaatcaggtcagcctcacctgtctcgtgaaaggcttctaccctagcgacattgccgtagaatgggaaagcaacgggcaaccagaaaacaattataagacaacacctcccgttctcgatagtgacggaagtttcttcctgtatagcaaacttaccgtggataaatcaagatggcagcaaggtaatgtgtttagctgttcagtaatgcacgaagctctgcataaccactacacccaaaaatctttgtctctgtctccagggtgaaaacaaacaaaa

SEQ ID NO: 19 - DNA, 2960 bp, Artificial Sequence
  synthetic
  modified_base (1157)..(1157): SLIM regulatory element
  modified_base (2550)..(2550): SLIM regulatory element
ggttggccactccctctctgcgcgctcgctcgctcactgaggccgggcgaccaaaggtcgcccgacgcccgggctttgcccgggcggcctcagtgagcgagcgagcgcgcagagagggagtggccaactccatcactaggggttcctagatctgaattcggtacccctagttattaatagtaatcaattacggggtcattagttcatagcccatatatggagttccgcgttacataacttacggtaaatggcccgcctggctgaccgcccaacgacccccgcccattgacgtcaataatgacgtatgttcccatagtaacgccaatagggactttccattgacgtcaatgggtggactatttacggtaaactgcccacttggcagtacatcaagtgtatcatatgccaagtacgccccctattgacgtcaatgacggtaaatggcccgcctggcattatgcccagtacatgaccttatgggactttcctacttggcagtacatctacgtattagtcatcgctattaccatggtcgaggtgagccccacgttctgcttcactctccccatctcccccccctccccacccccaattttgtatttatttattttttaattattttgtgcagcgatgggggcggggggggggggggggcgcgcgccaggcggggcggggcggggcgaggggcggggcggggcgaggcggagaggtgcggcggcagccaatcagagcggcgcgctccgaaagtttccttttatggcgaggcggcggcggcggcggccctataaaaagcgaagcgcgcggcgggcgggagtcgctgcgacgctgccttcgccccgtgccccgctccgccgccgcctcgcgccgcccgccccggctctgactgaccgcgttactcccacaggtgagcgggcgggacggcccttctcctccgggctgtaattagcgcttggtttaatgacggcttgtttcttttctgtggctgcgtgaaagccttgaggggctccgggagctagagcctctgctaaccatgttcatgccttcttctttttcctacagctcctgggcaacgtgctggttattgtgctgtctcatcattttggcaaagaattcctcgaagatctaggcaacgcgtctcgaggcggccgccgccaccaatggtatcatattgggacacaggagtcctcctgtgcgcccttttgagctgtcttttgctgacgggttcttcttcaggttctgataccgggagaccattcgttgaaatgtatagtgagatacccgaaattatacatatgactgaagggcgcgagctcgtcataccctgtcgggtaacaagtccaaacataacagtgaccctgaagaagttccctttggatactctcattcccgacgggaagcgaataatttgggactcaaggaagggatttatcatatctaatgcaacatataaggaaatagggctcctcacatgcgaagccacagtcaacgggcacctctacaaaactaattacctgacccatcgacagacaaataccatcattgatgtggttctgagtccatctcatggaatagagttgagtgtaggggagaagcttgttctcaattgcacagctagaaccgagttgaacgtgggtatcgattttaactgggaatacccatctagtaagcaccaacacaaaaaacttgtcaatcgagatttgaaaactcaatctggtagcgagatgaaaaagttcctgtcaactcttacaatcgatggcgtgacccggagtgatcaaggattgtatacctgcgccgccagctctggcctgatgactaaaaagaacagcacctttgtacgagtgcatgaaaaggataagactcatacatgccctccttgtcccgctccagagctgctgggaggtcccagtgttttcctcttcccaccaaagcccaaagatactctgatgattagccggacccctgaggtgacttgcgtcgtggtggatgtttcacatgaagatccagaagtgaagttcaattggtacgttgatggtgtggaggtacacaatgccaagactaaacctcgggaggaacagtataacagcacttacagagttgtcagcgtactcacagtgcttcatcaggactggttgaatggtaaggagtataagtgcaaagtgagtaataaggctctgccagcacccatagagaagacaatctcaaaggccaaaggccagccccgagaaccacaagtatacacactgccacctagtagagacgagttgacaaaaaatcaggtcagcctcacctgtctcgtgaaaggcttctaccctagcgacattgccgtagaatgggaaagcaacgggcaaccagaaaacaattataagacaacacctcccgttctcgatagtgacggaagtttcttcctgtatagcaaacttaccgtggataaatcaagatggcagcaaggtaatgtgtttagctgttcagtaatgcacgaagctctgcataaccactacacccaaaaatctttgtctctgtctccagggtgagcggccgcatcggctagcaaagcttcctgcaggagtcggtcgactagagctcgctgatcagcctcgactgtgccttctagttgccagccatctgttgtttgcccctcccccgtgccttccttgaccctggaaggtgccactcccactgtcctttcctaataaaatgaggaaattgcatcgcattgtctgagtaggtgtcattctattctggggggtggggtggggcaggacagcaagggggaggattgggaagacaatagcaggcatgctggggagagatctaggaacccctagtgatggagttggccactccctctctgcgcgctcgctcgctcactgaggccgcccgggcaaagcccgggcgtcgggcgacctttggtcgcccggcctcagtgagcgagcgagcgcgcagagagggagtggccaacc

SEQ ID NO: 20 - DNA, 1374 bp, Artificial Sequence; identical to SEQ ID NO: 8
  synthetic

SEQ ID NO: 21 - DNA, 153 bp, Artificial Sequence
  synthetic
gaacgcctcctaacgtctggtcacgaccctgcgtgagcgaccccattgttcaggtttgtattcttttggccactgactgagaatacaaatgaacaatgggggcgcctacgcagcccctcgaaatcacgagggagacgagataagggggcgttt

SEQ ID NO: 22 - DNA, 155 bp, Artificial Sequence
  synthetic
gaacgcctcctaacgtctggtcacgaccctgcgtgagcgaccctgagttccttccctaaatacttttggccactgactgagtatttaggaggaactcaggggggcgcctacgcagcccctcgaaatcacgagggagacgagataagggggcgttt

SEQ ID NO: 23 - DNA, 155 bp, Artificial Sequence
  synthetic
gaacgcctcctaacgtctggtcacgaccctgcgtgagcgaccaagagttaacgtgtcgatctcttttggccactgactgagagatcgacgttaactcttgggggcgcctacgcagcccctcgaaatcacgagggagacgagataagggggcgttt

SEQ ID NO: 24 - DNA, 155 bp, Artificial Sequence
  synthetic
gaacgcctcctaacgtctggtcacgaccctgcgtgagcgacccttccctaaatagtatagatcttttggccactgactgagatctatactttagggaaggggggcgcctacgcagcccctcgaaatcacgagggagacgagataagggggcgttt

SEQ ID NO: 25 - DNA, 155 bp, Artificial Sequence
  synthetic
gaacgcctcctaacgtctggtcacgaccctgcgtgagcgaccgtgtcgatcttggctcaactcttttggccactgactgagcgtgtcgattggctcaactggggcgcctacgcagcccctcgaaatcacgagggagacgagataagggggcgttt

SEQ ID NO: 26 - DNA, 127 bp, Artificial Sequence
  synthetic
gaacgcctccttgataccagctgcgtgagcgaccccattgttcaggtttgtattcttttggccactgactgagaatacaaatgaacaatgggggcgcctacgcgcccttggcagcaagggggcgttt

SEQ ID NO: 27 - DNA, 129 bp, Artificial Sequence
  synthetic
gaacgcctccttgataccagctgcgtgagcgaccctgagttccttccctaaatacttttggccactgactgagtatttaggaggaactcaggggggcgcctacgcgcccttggcagcaagggggcgttt

SEQ ID NO: 28 - DNA, 129 bp, Artificial Sequence
  synthetic
gaacgcctccttgataccagctgcgtgagcgaccaagagttaacgtgtcgatctcttttggccactgactgagagatcgacgttaactcttgggggcgcctacgcgcccttggcagcaagggggcgttt

SEQ ID NO: 29 - DNA, 129 bp, Artificial Sequence
  synthetic
gaacgcctccttgataccagctgcgtgagcgacccttccctaaatagtatagatcttttggccactgactgagatctatactttagggaaggggggcgcctacgcgcccttggcagcaagggggcgttt

SEQ ID NO: 30 - DNA, 129 bp, Artificial Sequence
  synthetic
gaacgcctccttgataccagctgcgtgagcgaccgtgtcgatcttggctcaactcttttggccactgactgagcgtgtcgattggctcaactggggcgcctacgcgcccttggcagcaagggggcgttt

SEQ ID NO: 31 - DNA, 151 bp, Artificial Sequence
  synthetic
gaacgcctcctagaggtgaagaatacgaccaccttgcgtgagcgaccccattgttcaggtttgtattcttttggccactgactgagaatacaaatgaacaatgggggcgcctacgcaggctcgaaagagcctaaaacataagggggcgttt

SEQ ID NO: 32 - DNA, 153 bp, Artificial Sequence
  synthetic
gaacgcctcctagaggtgaagaatacgaccaccttgcgtgagcgaccctgagttccttccctaaatacttttggccactgactgagtatttaggaggaactcaggggggcgcctacgcaggctcgaaagagcctaaaacataagggggcgttt

SEQ ID NO: 33 - DNA, 153 bp, Artificial Sequence
  synthetic
gaacgcctcctagaggtgaagaatacgaccaccttgcgtgagcgaccaagagttaacgtgtcgatctcttttggccactgactgagagatcgacgttaactcttgggggcgcctacgcaggctcgaaagagcctaaaacataagggggcgttt

SEQ ID NO: 34 - DNA, 153 bp, Artificial Sequence
  synthetic
gaacgcctcctagaggtgaagaatacgaccaccttgcgtgagcgacccttccctaaatagtatagatcttttggccactgactgagatctatactttagggaaggggggcgcctacgcaggctcgaaagagcctaaaacataagggggcgttt

SEQ ID NO: 35 - DNA, 153 bp, Artificial Sequence
  synthetic
gaacgcctcctagaggtgaagaatacgaccaccttgcgtgagcgaccgtgtcgatcttggctcaactcttttggccactgactgagcgtgtcgattggctcaactggggcgcctacgcaggctcgaaagagcctaaaacataagggggcgttt

SEQ ID NO: 36 - DNA, 2077 bp, Artificial Sequence
  synthetic
  modified_base (1)..(1): SLIM regulatory element
  modified_base (2077)..(2077): SLIM regulatory element
aatggtcagctactgggacaccggggtcctgctgtgcgcgctgctcagctgtctgcttctcacaggatctagttcaggttcaaaattaaaagatcctgaactgagtttaaaaggcacccagcacatcatgcaagcaggccagacactgcatctccaatgcaggggggaagcagcccataaatggtctttgcctgaaatggtgagtaaggaaagcgaaaggctgagcataactaaatctgcctgtggaagaaatggcaaacaattctgcagtactttaaccttgaacacagctcaagcaaaccacactggcttctacagctgcaaatatctagctgtacctacttcaaagaagaaggaaacagaatctgcaatctatatatttattagtgatacaggtagacctttcgtagagatgtacagtgaaatccccgaaattatacacatgactgaaggaagggagctcgtcattccctgccgggttacgtcacctaacatcactgttactttaaaaaagtttccacttgacactttgatccctgatggaaaacgcataatctgggacagtagaaagggcttcatcatatcaaatgcaacgtacaaagaaatagggcttctgacctgtgaagcaacagtcaatgggcatttgtataagacaaactatctcacacatcgacaaaccaatacaatcatagatgtccaaataagcacaccacgcccagtcaaattacttagaggccatactcttgtcctcaattgtactgctaccactcccttgaacacgagagttcaaatgacctggagttaccctgatgaaaaaaataagagagcttccgtaaggcgacgaattgaccaaagcaattcccatgccaacatattctacagtgttcttactattgacaaaatgcagaacaaagacaaaggactttatacttgtcgtgtaaggagtggaccatcattcaaatctgttaacacctcagtgcatatatatgataaagcattcatcactgtgaaacatcgaaaacagcaggtgcttgaaaccgtagctggcaagcggtcttaccggctctctatgaaagtgaaggcatttccctcgccggaagttgtatggttaaaagatgggttacctgcgactgagaaatctgctcgctatttgactcgtggctactcgttaattatcaaggacgtaactgaagaggatgcagggaattatacaatcttgctgagcataaaacagtcaaatgtgtttaaaaacctcactgccactctaattgtcaatgtgaaaccccagatttacgaaaaggccgtgtcatcgtttccagacccggctctctacccactgggcagcagacaaatcctgacttgtaccgcatatggtatccctcaacctacaatcaagtggttctggcacccctgtaaccataatcattccgaagcaaggtgtgacttttgttccaataatgaagagtcctttatcctggatgctgacagcaacatgggaaacagaattgagagcatcactcagcgcatggcaataatagaaggaaagaataagatggctagcaccttggttgtggctgactctagaatttctggaatctacatttgcatagcttccaataaagttgggactgtgggaagaaacataagcttttatatcacagatgtgccaaatgggtttcatgttaacttggaaaaaatgccgacggaaggagaggacctgaaactgtcttgcacagttaacaagttcttatacagagacgttacttggattttactgcggacagttaataacagaacaatgcactacagtattagcaagcaaaaaatggccatcactaaggagcactccatcactcttaatcttaccatcatgaatgtttccctgcaagattcaggcacctatgcctgcagagccaggaatgtatacacaggggaagaaatcctccagaagaaagaaattacaatcagaggtgagcactgcaacaaaaaggctgttttctctcggatctccaaatttaaaagcacaaggaatgattgtaccacacaaagtaatgtaaaacattaaaaacaaacaaaa

SEQ ID NO: 37 - DNA, 155 bp, Artificial Sequence
  synthetic
gaacgcctcctaacgtctggtcacgaccctgcgtgagcgaccagacgaagagtgtcctagatcttttggccactgactgagatctaggactcttcgtctgggggcgcctacgcagcccctcgaaatcacgagggagacgagataagggggcgttt

SEQ ID NO: 38 - DNA, 155 bp, Artificial Sequence
  synthetic
gaacgcctcctaacgtctggtcacgaccctgcgtgagcgaccgctttccgactcgtattgatcttttggccactgactgagatcaatacgtcggaaagcgggggcgcctacgcagcccctcgaaatcacgagggagacgagataagggggcgttt

SEQ ID NO: 39 - DNA, 155 bp, Artificial Sequence
  synthetic
gaacgcctcctaacgtctggtcacgaccctgcgtgagcgaccaccttctttaccgtttgttacttttggccactgactgagtaacaaactaaagaaggtgggggcgcctacgcagcccctcgaaatcacgagggagacgagataagggggcgttt

SEQ ID NO: 40 - DNA, 155 bp, Artificial Sequence
  synthetic
gaacgcctcctaacgtctggtcacgaccctgcgtgagcgacccgtttgttaagacgtcatgacttttggccactgactgagtcatgacgttaacaaacggggggcgcctacgcagcccctcgaaatcacgagggagacgagataagggggcgttt

SEQ ID NO: 41 - DNA, 155 bp, Artificial Sequence
  synthetic
gaacgcctcctaacgtctggtcacgaccctgcgtgagcgacgcaaatatctagctgtacctacttttggccactgactgagtaggtacatagatatttgcggggcgcctacgcagcccctcgaaatcacgagggagacgagataagggggcgttt

SEQ ID NO: 42 - DNA, 129 bp, Artificial Sequence
  synthetic
gaacgcctccttgataccagctgcgtgagcgaccagacgaagagtgtcctagatcttttggccactgactgagatctaggactcttcgtctgggggcgcctacgcgcccttggcagcaagggggcgttt

SEQ ID NO: 43 - DNA, 129 bp, Artificial Sequence
  synthetic
gaacgcctccttgataccagctgcgtgagcgaccgctttccgactcgtattgatcttttggccactgactgagatcaatacgtcggaaagcgggggcgcctacgcgcccttggcagcaagggggcgttt

SEQ ID NO: 44 - DNA, 129 bp, Artificial Sequence
  synthetic
gaacgcctccttgataccagctgcgtgagcgaccaccttctttaccgtttgttacttttggccactgactgagtaacaaactaaagaaggtgggggcgcctacgcgcccttggcagcaagggggcgttt

SEQ ID NO: 45 - DNA, 129 bp, Artificial Sequence
  synthetic
gaacgcctccttgataccagctgcgtgagcgacccgtttgttaagacgtcatgacttttggccactgactgagtcatgacgttaacaaacggggggcgcctacgcgcccttggcagcaagggggcgttt

SEQ ID NO: 46 - DNA, 129 bp, Artificial Sequence
  synthetic
gaacgcctccttgataccagctgcgtgagcgacgcaaatatctagctgtacctacttttggccactgactgagtaggtacatagatatttgcggggcgcctacgcgcccttggcagcaagggggcgttt

SEQ ID NO: 47 - DNA, 153 bp, Artificial Sequence
  synthetic
gaacgcctcctagaggtgaagaatacgaccaccttgcgtgagcgaccagacgaagagtgtcctagatcttttggccactgactgagatctaggactcttcgtctgggggcgcctacgcaggctcgaaagagcctaaaacataagggggcgttt

SEQ ID NO: 48 - DNA, 153 bp, Artificial Sequence
  synthetic
gaacgcctcctagaggtgaagaatacgaccaccttgcgtgagcgaccgctttccgactcgtattgatcttttggccactgactgagatcaatacgtcggaaagcgggggcgcctacgcaggctcgaaagagcctaaaacataagggggcgttt

SEQ ID NO: 49 - DNA, 153 bp, Artificial Sequence
  synthetic
gaacgcctcctagaggtgaagaatacgaccaccttgcgtgagcgaccaccttctttaccgtttgttacttttggccactgactgagtaacaaactaaagaaggtgggggcgcctacgcaggctcgaaagagcctaaaacataagggggcgttt

SEQ ID NO: 50 - DNA, 153 bp, Artificial Sequence
  synthetic
gaacgcctcctagaggtgaagaatacgaccaccttgcgtgagcgacccgtttgttaagacgtcatgacttttggccactgactgagtcatgacgttaacaaacggggggcgcctacgcaggctcgaaagagcctaaaacataagggggcgttt

SEQ ID NO: 51 - DNA, 142 bp, Artificial Sequence
  synthetic
gaacgcctcctagaggtgaagaatacgaccaccttgcgtgagcgacgcaaatatctagctgtacctacttttggccactgactgagtaggtacatagatatttgcggggcgcctacgcaggctcgaaagagcctaaaacata

SEQ ID NO: 52 - DNA, 1815 bp, Artificial Sequence
  synthetic
atgcttgcccgggccctgcttctgtgtgcggtattggcactgagtcacacagccaacccgtgctgctcacacccatgtcagaatcggggagtttgcatgtcagtagggtttgaccaatataagtgcgactgtacccggacaggcttttatggagaaaattgttctacacccgaatttttgacgaggattaagctctttctgaagcctacaccaaatacagtccattatatcctcacgcacttcaagggtttttggaatgtcgtaaacaacattccgtttctgagaaatgcgataatgtcttacgtccttacatcccggagccaccttattgactcacccccaacatacaacgccgactacggatacaaaagttgggaagctttctccaacctgtcttactacacgcgagcattgcctcctgtacccgacgattgcccgacgccgttgggggtgaaaggaaaaaagcagctcccggactcaaacgaaatagtagagaaattgttgcttcgccgaaaatttataccagacccgcagggtagcaatatgatgtttgcgttcttcgctcagcacttcactcaccaattctttaagacagaccacaagagaggtcccgcattcacgaatggccttggacacggcgtcgacttgaaccacatatatggggagacattggccagacaaaggaaacttcgattgtttaaggatgggaaaatgaaataccaaattattgatggcgagatgtatcctccaacagtgaaggatacgcaagcggagatgatttatccaccgcaggtaccagagcatttgcggttcgcggtggggcaggaagtatttggacttgttcccggtctgatgatgtacgccacaatatggctccgggagcataatcgcgtgtgtgacgtacttaagcaagagcacccggaatggggcgacgagcaactttttcaaacgagtcgactgattctcattggggaaacgattaaaatagtgatcgaagattatgtgcaacatctttctggttaccactttaagttgaagttcgatcctgagctgcttttcaataaacaattccagtatcaaaacagaatcgccgcggagttcaacacgctgtatcattggcatcccctgttgcccgatacttttcaaatccatgaccagaaatacaattaccagcaatttatatataataactctatcctcctggagcatggcattacacaattcgttgaaagtttcacaaggcagatcgcaggaagagttgcgggtggccggaatgtgccgcctgccgtgcaaaaggtatcacaggctagcatcgaccaatcaaggcaaatgaagtaccagtcttttaatgagtacaggaaaaggttcatgctgaagccttacgagagctttgaagaactgacgggcgaaaaggaaatgtccgcggaactggaagcgttgtacggagatattgatgcggtagagctctaccccgcgcttctggtcgaaaagccccggccagatgccattttcggggaaaccatggttgaagtgggcgccccattcagtttgaaaggtctgatgggtaatgtaatttgcagtccggcgtactggaagccttccacttttggtggggaagtggggtttcaaattatcaatacggcctcaattcagtctctgatttgtaacaatgttaagggatgtccctttacatcttttagtgtaccggaccccgagcttattaagaccgtgaccataaatgcttcaagctctagaagtggtcttgatgatatcaaccccacagttttgcttaaggaaaggagcacggagctctaa

SEQ ID NO: 53 - DNA, 894 bp, Artificial Sequence
  synthetic
atgagcatgaacaactcaaaacagttggtctccccagcagcggcccttttgtccaacacaacgtgtcagactgagaatagactcagtgtattttttagcgtgatttttatgaccgtcggtatcctgtctaactctcttgccatagcaatattgatgaaagcctatcagcgattccggcaaaagtctaaggcgtcatttttgttgttggcaagcgggcttgtcatcacggactttttcgggcacctcattaacggagccatagccgtgttcgtttatgcttcagacaaagagtggatacgattcgatcagagcaatgtgctttgcagtatctttggcatatgtatggtgtttagtggattgtgtccactcttgcttgggagcgtgatggctattgaaagatgcatcggggtgactaaacctatctttcacagtaccaaaattacatctaagcacgtcaagatgatgttgtccggggtgtgtctttttgctgtctttattgcgttgttgccaatactgggccacagggactacaaaattcaggcctcacgcacttggtgcttctataacactgaggatattaaagactgggaggataggttttatcttcttcttttctcattcctcggtctgctcgcactgggggtatcccttttgtgtaacgctatcacaggtatcaccttgttgcgcgttaaatttaagagccaacagcatcgccaggggaggtcacatcacctcgaaatggtaatacagttgctcgcgatcatgtgtgttagttgtatctgctggtcacccttcttgggatatagaataattctgaatggaaaagaaaagtacaaagtctatgaagaacagagcgattttctgcatcgattgcaatggcccactttggaataa

SEQ ID NO: 54 - DNA, 2771 bp, Artificial Sequence
  synthetic
  modified_base (1)..(1): SLIM regulatory element
  modified_base (2771)..(2771): SLIM regulatory element
aatgcttgcccgggccctgcttctgtgtgcggtattggcactgagtcacacagccaacccgtgctgctcacacccatgtcagaatcggggagtttgcatgtcagtagggtttgaccaatataagtgcgactgtacccggacaggcttttatggagaaaattgttctacacccgaatttttgacgaggattaagctctttctgaagcctacaccaaatacagtccattatatcctcacgcacttcaagggtttttggaatgtcgtaaacaacattccgtttctgagaaatgcgataatgtcttacgtccttacatcccggagccaccttattgactcacccccaacatacaacgccgactacggatacaaaagttgggaagctttctccaacctgtcttactacacgcgagcattgcctcctgtacccgacgattgcccgacgccgttgggggtgaaaggaaaaaagcagctcccggactcaaacgaaatagtagagaaattgttgcttcgccgaaaatttataccagacccgcagggtagcaatatgatgtttgcgttcttcgctcagcacttcactcaccaattctttaagacagaccacaagagaggtcccgcattcacgaatggccttggacacggcgtcgacttgaaccacatatatggggagacattggccagacaaaggaaacttcgattgtttaaggatgggaaaatgaaataccaaattattgatggcgagatgtatcctccaacagtgaaggatacgcaagcggagatgatttatccaccgcaggtaccagagcatttgcggttcgcggtggggcaggaagtatttggacttgttcccggtctgatgatgtacgccacaatatggctccgggagcataatcgcgtgtgtgacgtacttaagcaagagcacccggaatggggcgacgagcaactttttcaaacgagtcgactgattctcattggggaaacgattaaaatagtgatcgaagattatgtgcaacatctttctggttaccactttaagttgaagttcgatcctgagctgcttttcaataaacaattccagtatcaaaacagaatcgccgcggagttcaacacgctgtatcattggcatcccctgttgcccgatacttttcaaatccatgaccagaaatacaattaccagcaatttatatataataactctatcctcctggagcatggcattacacaattcgttgaaagtttcacaaggcagatcgcaggaagagttgcgggtggccggaatgtgccgcctgccgtgcaaaaggtatcacaggctagcatcgaccaatcaaggcaaatgaagtaccagtcttttaatgagtacaggaaaaggttcatgctgaagccttacgagagctttgaagaactgacgggcgaaaaggaaatgtccgcggaactggaagcgttgtacggagatattgatgcggtagagctctaccccgcgcttctggtcgaaaagccccggccagatgccattttcggggaaaccatggttgaagtgggcgccccattcagtttgaaaggtctgatgggtaatgtaatttgcagtccggcgtactggaagccttccacttttggtggggaagtggggtttcaaattatcaatacggcctcaattcagtctctgatttgtaacaatgttaagggatgtccctttacatcttttagtgtaccggaccccgagcttattaagaccgtgaccataaatgcttcaagctctagaagtggtcttgatgatatcaaccccacagttttgcttaaggaaaggagcacggagctcggaagcggagctactaacttcagcctgctgaagcaggctggagacgtcgaggagaaccctggacctagcatgaacaactcaaaacagttggtctccccagcagcggcccttttgtccaacacaacgtgtcagactgagaatagactcagtgtattttttagcgtgatttttatgaccgtcggtatcctgtctaactctcttgccatagcaatattgatgaaagcctatcagcgattccggcaaaagtctaaggcgtcatttttgttgttggcaagcgggcttgtcatcacggactttttcgggcacctcattaacggagccatagccgtgttcgtttatgcttcagacaaagagtggatacgattcgatcagagcaatgtgctttgcagtatctttggcatatgtatggtgtttagtggattgtgtccactcttgcttgggagcgtgatggctattgaaagatgcatcggggtgactaaacctatctttcacagtaccaaaattacatctaagcacgtcaagatgatgttgtccggggtgtgtctttttgctgtctttattgcgttgttgccaatactgggccacagggactacaaaattcaggcctcacgcacttggtgcttctataacactgaggatattaaagactgggaggataggttttatcttcttcttttctcattcctcggtctgctcgcactgggggtatcccttttgtgtaacgctatcacaggtatcaccttgttgcgcgttaaatttaagagccaacagcatcgccaggggaggtcacatcacctcgaaatggtaatacagttgctcgcgatcatgtgtgttagttgtatctgctggtcacccttcttgggatatagaataattctgaatggaaaagaaaagtacaaagtctatgaagaacagagcgattttctgcatcgattgcaatggcccactttggaataaa

SEQ ID NO: 55 - DNA, 1812 bp, Artificial Sequence
  synthetic
atgcttgcccgggccctgcttctgtgtgcggtattggcactgagtcacacagccaacccgtgctgctcacacccatgtcagaatcggggagtttgcatgtcagtagggtttgaccaatataagtgcgactgtacccggacaggcttttatggagaaaattgttctacacccgaatttttgacgaggattaagctctttctgaagcctacaccaaatacagtccattatatcctcacgcacttcaagggtttttggaatgtcgtaaacaacattccgtttctgagaaatgcgataatgtcttacgtccttacatcccggagccaccttattgactcacccccaacatacaacgccgactacggatacaaaagttgggaagctttctccaacctgtcttactacacgcgagcattgcctcctgtacccgacgattgcccgacgccgttgggggtgaaaggaaaaaagcagctcccggactcaaacgaaatagtagagaaattgttgcttcgccgaaaatttataccagacccgcagggtagcaatatgatgtttgcgttcttcgctcagcacttcactcaccaattctttaagacagaccacaagagaggtcccgcattcacgaatggccttggacacggcgtcgacttgaaccacatatatggggagacattggccagacaaaggaaacttcgattgtttaaggatgggaaaatgaaataccaaattattgatggcgagatgtatcctccaacagtgaaggatacgcaagcggagatgatttatccaccgcaggtaccagagcatttgcggttcgcggtggggcaggaagtatttggacttgttcccggtctgatgatgtacgccacaatatggctccgggagcataatcgcgtgtgtgacgtacttaagcaagagcacccggaatggggcgacgagcaactttttcaaacgagtcgactgattctcattggggaaacgattaaaatagtgatcgaagattatgtgcaacatctttctggttaccactttaagttgaagttcgatcctgagctgcttttcaataaacaattccagtatcaaaacagaatcgccgcggagttcaacacgctgtatcattggcatcccctgttgcccgatacttttcaaatccatgaccagaaatacaattaccagcaatttatatataataactctatcctcctggagcatggcattacacaattcgttgaaagtttcacaaggcagatcgcaggaagagttgcgggtggccggaatgtgccgcctgccgtgcaaaaggtatcacaggctagcatcgaccaatcaaggcaaatgaagtaccagtcttttaatgagtacaggaaaaggttcatgctgaagccttacgagagctttgaagaactgacgggcgaaaaggaaatgtccgcggaactggaagcgttgtacggagatattgatgcggtagagctctaccccgcgcttctggtcgaaaagccccggccagatgccattttcggggaaaccatggttgaagtgggcgccccattcagtttgaaaggtctgatgggtaatgtaatttgcagtccggcgtactggaagccttccacttttggtggggaagtggggtttcaaattatcaatacggcctcaattcagtctctgatttgtaacaatgttaagggatgtccctttacatcttttagtgtaccggaccccgagcttattaagaccgtgaccataaatgcttcaagctctagaagtggtcttgatgatatcaaccccacagttttgcttaaggaaaggagcacggagctc

SEQ ID NO: 56 - DNA, 66 bp, Artificial Sequence
  synthetic
ggaagcggagctactaacttcagcctgctgaagcaggctggagacgtcgaggagaaccctggacct

SEQ ID NO: 57 - DNA, 891 bp, Artificial Sequence
  synthetic
agcatgaacaactcaaaacagttggtctccccagcagcggcccttttgtccaacacaacgtgtcagactgagaatagactcagtgtattttttagcgtgatttttatgaccgtcggtatcctgtctaactctcttgccatagcaatattgatgaaagcctatcagcgattccggcaaaagtctaaggcgtcatttttgttgttggcaagcgggcttgtcatcacggactttttcgggcacctcattaacggagccatagccgtgttcgtttatgcttcagacaaagagtggatacgattcgatcagagcaatgtgctttgcagtatctttggcatatgtatggtgtttagtggattgtgtccactcttgcttgggagcgtgatggctattgaaagatgcatcggggtgactaaacctatctttcacagtaccaaaattacatctaagcacgtcaagatgatgttgtccggggtgtgtctttttgctgtctttattgcgttgttgccaatactgggccacagggactacaaaattcaggcctcacgcacttggtgcttctataacactgaggatattaaagactgggaggataggttttatcttcttcttttctcattcctcggtctgctcgcactgggggtatcccttttgtgtaacgctatcacaggtatcaccttgttgcgcgttaaatttaagagccaacagcatcgccaggggaggtcacatcacctcgaaatggtaatacagttgctcgcgatcatgtgtgttagttgtatctgctggtcacccttcttgggatatagaataattctgaatggaaaagaaaagtacaaagtctatgaagaacagagcgattttctgcatcgattgcaatggcccactttggaataa

SEQ ID NO: 58 - DNA, 4621 bp, Artificial Sequence
  synthetic
ggttggccactccctctctgcgcgctcgctcgctcactgaggccgggcgaccaaaggtcgcccgacgcccgggctttgcccgggcggcctcagtgagcgagcgagcgcgcagagagggagtggccaactccatcactaggggttcctagatctgaattcggtacccctagttattaatagtaatcaattacggggtcattagttcatagcccatatatggagttccgcgttacataacttacggtaaatggcccgcctggctgaccgcccaacgacccccgcccattgacgtcaataatgacgtatgttcccatagtaacgccaatagggactttccattgacgtcaatgggtggactatttacggtaaactgcccacttggcagtacatcaagtgtatcatatgccaagtacgccccctattgacgtcaatgacggtaaatggcccgcctggcattatgcccagtacatgaccttatgggactttcctacttggcagtacatctacgtattagtcatcgctattaccatggtcgaggtgagccccacgttctgcttcactctccccatctcccccccctccccacccccaattttgtatttatttattttttaattattttgtgcagcgatgggggcggggggggggggggggcgcgcgccaggcggggcggggcggggcgaggggcggggcggggcgaggcggagaggtgcggcggcagccaatcagagcggcgcgctccgaaagtttccttttatggcgaggcggcggcggcggcggccctataaaaagcgaagcgcgcggcgggcgggagtcgctgcgacgctgccttcgccccgtgccccgctccgccgccgcctcgcgccgcccgccccggctctgactgaccgcgttactcccacaggtgagcgggcgggacggcccttctcctccgggctgtaattagcgcttggtttaatgacggcttgtttcttttctgtggctgcgtgaaagccttgaggggctccgggagctagagcctctgctaaccatgttcatgccttcttctttttcctacagctcctgggcaacgtgctggttattgtgctgtctcatcattttggcaaagaattcctcgaagatctaggcaactcgagaaacaaacaaactgaggtgcaggtacatccagctgacgagtcccaaataggacgaaagggagaggtgaagaatacgaccacctaggctcgaaagagcctaaaacataccttcctggattccactgctatccacaaaaagaaaaataaaaagccaccatgcttgcccgggccctgcttctgtgtgcggtattggcactgagtcacacagccaacccgtgctgctcacacccatgtcagaatcggggagtttgcatgtcagtagggtttgaccaatataagtgcgactgtacccggacaggcttttatggagaaaattgttctacacccgaatttttgacgaggattaagctctttctgaagcctacaccaaatacagtccattatatcctcacgcacttcaagggtttttggaatgtcgtaaacaacattccgtttctgagaaatgcgataatgtcttacgtccttacatcccggagccaccttattgactcacccccaacatacaacgccgactacggatacaaaagttgggaagctttctccaacctgtcttactacacgcgagcattgcctcctgtacccgacgattgcccgacgccgttgggggtgaaaggaaaaaagcagctcccggactcaaacgaaatagtagagaaattgttgcttcgccgaaaatttataccagacccgcagggtagcaatatgatgtttgcgttcttcgctcagcacttcactcaccaattctttaagacagaccacaagagaggtcccgcattcacgaatggccttggacacggcgtcgacttgaaccacatatatggggagacattggccagacaaaggaaacttcgattgtttaaggatgggaaaatgaaataccaaattattgatggcgagatgtatcctccaacagtgaaggatacgcaagcggagatgatttatccaccgcaggtaccagagcatttgcggttcgcggtggggcaggaagtatttggacttgttcccggtctgatgatgtacgccacaatatggctccgggagcataatcgcgtgtgtgacgtacttaagcaagagcacccggaatggggcgacgagcaactttttcaaacgagtcgactgattctcattggggaaacgattaaaatagtgatcgaagattatgtgcaacatctttctggttaccactttaagttgaagttcgatcctgagctgcttttcaataaacaattccagtatcaaaacagaatcgccgcggagttcaacacgctgtatcattggcatcccctgttgcccgatacttttcaaatccatgaccagaaatacaattaccagcaatttatatataataactctatcctcctggagcatggcattacacaattcgttgaaagtttcacaaggcagatcgcaggaagagttgcgggtggccggaatgtgccgcctgccgtgcaaaaggtatcacaggctagcatcgaccaatcaaggcaaatgaagtaccagtcttttaatgagtacaggaaaaggttcatgctgaagccttacgagagctttgaagaactgacgggcgaaaaggaaatgtccgcggaactggaagcgttgtacggagatattgatgcggtagagctctaccccgcgcttctggtcgaaaagccccggccagatgccattttcggggaaaccatggttgaagtgggcgccccattcagtttgaaaggtctgatgggtaatgtaatttgcagtccggcgtactggaagccttccacttttggtggggaagtggggtttcaaattatcaatacggcctcaattcagtctctgatttgtaacaatgttaagggatgtccctttacatcttttagtgtaccggaccccgagcttattaagaccgtgaccataaatgcttcaagctctagaagtggtcttgatgatatcaaccccacagttttgcttaaggaaaggagcacggagctcggaagcggagctactaacttcagcctgctgaagcaggctggagacgtcgaggagaaccctggacctagcatgaacaactcaaaacagttggtctccccagcagcggcccttttgtccaacacaacgtgtcagactgagaatagactcagtgtattttttagcgtgatttttatgaccgtcggtatcctgtctaactctcttgccatagcaatattgatgaaagcctatcagcgattccggcaaaagtctaaggcgtcatttttgttgttggcaagcgggcttgtcatcacggactttttcgggcacctcattaacggagccatagccgtgttcgtttatgcttcagacaaagagtggatacgattcgatcagagcaatgtgctttgcagtatctttggcatatgtatggtgtttagtggattgtgtccactcttgcttgggagcgtgatggctattgaaagatgcatcggggtgactaaacctatctttcacagtaccaaaattacatctaagcacgtcaagatgatgttgtccggggtgtgtctttttgctgtctttattgcgttgttgccaatactgggccacagggactacaaaattcaggcctcacgcacttggtgcttctataacactgaggatattaaagactgggaggataggttttatcttcttcttttctcattcctcggtctgctcgcactgggggtatcccttttgtgtaacgctatcacaggtatcaccttgttgcgcgttaaatttaagagccaacagcatcgccaggggaggtcacatcacctcgaaatggtaatacagttgctcgcgatcatgtgtgttagttgtatctgctggtcacccttcttgggatatagaataattctgaatggaaaagaaaagtacaaagtctatgaagaacagagcgattttctgcatcgattgcaatggcccactttggaataaaaacaaacaaactgagatgcaggtacatcccactgatgagtcccaaataggacgaaagggagaggtgaagaatacgaccacctaggctcgaaagagcctaaaacataccttctgggattccactgctatccacaaaaagaaaaataaaaagcggccgctgcaggagtcggtcgactagagctcgctgatcagcctcgactgtgccttctagttgccagccatctgttgtttgcccctcccccgtgccttccttgaccctggaaggtgccactcccactgtcctttcctaataaaatgaggaaattgcatcgcattgtctgagtaggtgtcattctattctggggggtggggtggggcaggacagcaagggggaggattgggaagacaatagcaggcatgctggggagagatctaggaacccctagtgatggagttggccactccctctctgcgcgctcgctcgctcactgaggccgcccgggcaaagcccgggcgtcgggcgacctttggtcgcccggcctcagtgagcgagcgagcgcgcagagagggagtggccaacc

SEQ ID NO: 59 - DNA, 122 bp, Artificial Sequence
  synthetic
ctgaggtgcaggtacatccagctgacgagtcccaaataggacgaaagggagaggtgaagaatacgaccacctaggctcgaaagagcctaaaacataccttcctggattccactgctatccac

SEQ ID NO: 60 - DNA, 1812 bp, Artificial Sequence; identical to SEQ ID NO: 55
  synthetic

SEQ ID NO: 61 - DNA, 66 bp, Artificial Sequence; identical to SEQ ID NO: 56
  synthetic

SEQ ID NO: 62 - DNA, 891 bp, Artificial Sequence; identical to SEQ ID NO: 57
  synthetic

SEQ ID NO: 63 - DNA, 122 bp, Artificial Sequence
  synthetic
ctgagatgcaggtacatcccactgatgagtcccaaataggacgaaagggagaggtgaagaatacgaccacctaggctcgaaagagcctaaaacataccttctgggattccactgctatccac

SEQ ID NO: 64 - DNA, 168 bp, Artificial Sequence; identical to SEQ ID NO: 11
  synthetic

SEQ ID NO: 65 - DNA, 139 bp, Artificial Sequence; identical to SEQ ID NO: 13
  synthetic

SEQ ID NO: 66 - DNA, 135 bp, Artificial Sequence; identical to SEQ ID NO: 14
  synthetic

SEQ ID NO: 67 - DNA, 134 bp, Artificial Sequence; identical to SEQ ID NO: 15
  synthetic

SEQ ID NO: 68 - DNA, 104 bp, Artificial Sequence
  synthetic
gagagaatcttctttctgtctataaaagagagaatcttctttctgtctataaaagagagaatcttctttctgtctataaaagagagaatcttctttctgtctat

SEQ ID NO: 69 - DNA, 124 bp, Artificial Sequence
  synthetic
gcggccgcgctagcacgggtcctgataccagcgtgagcggagagaatcttctttctgtctattagtgaagccacagatgtaatagacagaaagaagattctctccgcctacgcccttggcagca

SEQ ID NO: 70 - DNA, 21 bp, Artificial Sequence
  synthetic
tatttagggaaggaactcagg

SEQ ID NO: 71 - DNA, 21 bp, Artificial Sequence
  synthetic
aatacaaacctgaacaatggg

SEQ ID NO: 72 - DNA, 21 bp, Artificial Sequence
  synthetic
agttgagccaagatcgacacg

SEQ ID NO: 73 - DNA, 21 bp, Artificial Sequence
  synthetic
atctatactatttagggaagg

SEQ ID NO: 74 - DNA, 21 bp, Artificial Sequence
  synthetic
agatcgacacgttaactcttg

SEQ ID NO: 75 - DNA, 21 bp, Artificial Sequence
  synthetic
taggtacagctagatatttgc

SEQ ID NO: 76 - DNA, 21 bp, Artificial Sequence
  synthetic
tcatgacgtcttaacaaacgg

SEQ ID NO: 77 - DNA, 21 bp, Artificial Sequence
  synthetic
taacaaacggtaaagaaggtg

SEQ ID NO: 78 - DNA, 21 bp, Artificial Sequence
  synthetic
atcaatacgagtcggaaagcg

SEQ ID NO: 79 - DNA, 21 bp, Artificial Sequence
  synthetic
atctaggacactcttcgtctg